European Patent Application EP 4 756 018 A1, published June 10, 2026. Title: Novel bifunctional glutamate N-acetyltransferase/amino-acid acetyltransferase variant and a method for producing glutamate family amino acids using the same. Applicant: CJ CheilJedang Corporation. Application KR. The sequence listing filed with the application follows.

SEQUENCE LISTING (52 sequences)

SEQ ID NO: 1 - protein, 388 aa, Corynebacterium glutamicum
MAKKGITAPKGFVASATTAGIKASGNPDMALVVNQGPEFSAAAVFTRNRVFAAPVKVSRENVADGQIRAVLYNAGNANACNGLQGEKDARESVSHLAQNLGLEDSDIGVCSTGLIGELLPMDKLNTGIDQLTAEGALGDNGAAAAKAIMTTDTVDKETVVFADGWTVGGMGKGVGMMAPSLATMLVCLTTDASVTQEMAQIALANATAVTFDTLDIDGSTSTNDTVFLLASGASGITPTQDELNDAVYAACSDIAAKLQADAEGVTKRVAVTVVGTTNNEQAINAARTVARDNLFKCAMFGSDPNWGRVLAAVGMADADMEPEKISVFFNDQAVCLDSTGAPGAREVDLSGADIDVRIDLGTSGEGQATVRTTDLSFSYVEINSAYSS

SEQ ID NO: 2 - DNA, 1167 bp, Corynebacterium glutamicum
  source 1..1167: mol_type = genomic DNA
atggccaaaaaaggcattaccgcgccgaaaggcttcgttgcttctgcaacgaccgcgggtattaaagcttctggcaatcctgacatggcgttggtggttaaccagggtccagagttttccgcagcggccgtgtttacacgcaaccgagttttcgcagcgcctgtgaaggtgagccgggagaacgttgctgatggccagatcagggctgttttgtacaacgctggtaatgctaatgcgtgtaatggtctgcagggtgagaaggatgctcgtgagtctgtttctcatctagctcaaaatttgggcttggaggattccgatattggtgtgtgttccactggtcttattggtgagttgcttccgatggataagctcaatacaggtattgatcagctgaccgctgagggcgctttgggtgacaatggtgcagctgctgccaaggcgatcatgaccactgacacggtggataaggaaaccgtcgtgtttgctgatggttggactgtcggcggaatgggcaagggcgtgggcatgatggcgccgtctcttgccaccatgctggtctgcttgaccactgatgcatccgttactcaggaaatggctcagattgcgctggctaatgctacggccgttacgtttgacaccctggatattgatggatcaacctccaccaatgacaccgtgttcctgctggcatctggcgctagcggaatcaccccaactcaggatgaactcaacgatgcggtgtacgcagcttgttctgatatcgcagcgaagcttcaggctgatgcagagggggtgaccaagcgcgttgctgtgacagtggtgggaaccaccaacaacgagcaggcgatcaatgcggctcgcacggttgctcgtgacaatttgttcaagtgcgcaatgtttggatctgatccaaactggggtcgcgtgttggctgcagtcggcatggctgatgctgatatggaaccagagaagatttctgtgttcttcaatgatcaagcagtatgccttgattccactggcgctcctggtgctcgtgaggtggatctttccggcgctgacattgatgtccgaattgatttgggcaccagtggggaaggccaggcaacagttcgaaccactgacctgagcttctcctacgtggagatcaactccgcgtacagctcttaa

SEQ ID NO: 3 - protein, 388 aa, synthetic construct
MAKKGITAPKGFVASATTAGIKASGNPDMALVVNQGPEFSAAAVFTRNRVFAAPVKVSRENVADGQIRAVLYNAGNANACNGLQGEKDARESVSHLAQNLGLEDSDIGVCSTGLIGELLPMDKLNTGIDQLTAEGALGDNGAAAAKAIMTTDTVDKETVVFADGWTVGGMGKGVGMMAPSLATMLVCLTTDASVTQEMAQFALANATAVTFDTLDIDGSTSTNDTVFLLASGASGITPTQDELNDAVYAACSDIAAKLQADAEGVTKRVAVTVVGTTNNEQAINAARTVARDNLFKCAMFGSDPNWGRVLAAVGMADADMEPEKISVFFNDQAVCLDSTGAPGAREVDLSGADIEVRIDLGTSGEGQATVRTTDLSFSYVEINSAYSS

SEQ ID NO: 4 - DNA, 1167 bp, synthetic construct
  source 1..1167: mol_type = other DNA
atggccaaaaaaggcattaccgcgccgaaaggcttcgttgcttctgcaacgaccgcgggtattaaagcttctggcaatcctgacatggcgttggtggttaaccagggtccagagttttccgcagcggccgtgtttacacgcaaccgagttttcgcagcgcctgtgaaggtgagccgggagaacgttgctgatggccagatcagggctgttttgtacaacgctggtaatgctaatgcgtgtaatggtctgcagggtgagaaggatgctcgtgagtctgtttctcatctagctcaaaatttgggcttggaggattccgatattggtgtgtgttccactggtcttattggtgagttgcttccgatggataagctcaatacaggtattgatcagctgaccgctgagggcgctttgggtgacaatggtgcagctgctgccaaggcgatcatgaccactgacacggtggataaggaaaccgtcgtgtttgctgatggttggactgtcggcggaatgggcaagggcgtgggcatgatggcgccgtctcttgccaccatgctggtctgcttgaccactgatgcatccgttactcaggaaatggctcagtttgcgctggctaatgctacggccgttacgtttgacaccctggatattgatggatcaacctccaccaatgacaccgtgttcctgctggcatctggcgctagcggaatcaccccaactcaggatgaactcaacgatgcggtgtacgcagcttgttctgatatcgcagcgaagcttcaggctgatgcagagggggtgaccaagcgcgttgctgtgacagtggtgggaaccaccaacaacgagcaggcgatcaatgcggctcgcacggttgctcgtgacaatttgttcaagtgcgcaatgtttggatctgatccaaactggggtcgcgtgttggctgcagtcggcatggctgatgctgatatggaaccagagaagatttctgtgttcttcaatgatcaagcagtatgccttgattccactggcgctcctggtgctcgtgaggtggatctttccggcgctgacattgaggtccgaattgatttgggcaccagtggggaaggccaggcaacagttcgaaccactgacctgagcttctcctacgtggagatcaactccgcgtacagctcttaa

SEQ ID NO: 5 - DNA, 34 bp, synthetic construct
  source 1..34: mol_type = other DNA
caaattcgaaaccgataatggccaaaaaaggcat

SEQ ID NO: 6 - DNA, 34 bp, synthetic construct
  source 1..34: mol_type = other DNA
cagcgcaaactgagccatttcctgagtaacggat

SEQ ID NO: 7 - DNA, 34 bp, synthetic construct
  source 1..34: mol_type = other DNA
tggctcagtttgcgctggctaatgctacggccgt

SEQ ID NO: 8 - DNA, 34 bp, synthetic construct
  source 1..34: mol_type = other DNA
caattcggacctcaatgtcagcgccggaaagatc

SEQ ID NO: 9 - DNA, 34 bp, synthetic construct
  source 1..34: mol_type = other DNA
cattgaggtccgaattgatttgggcaccagtggg

SEQ ID NO: 10 - DNA, 34 bp, synthetic construct
  source 1..34: mol_type = other DNA
gtggcggccgctctagattaagagctgtacgcgg

SEQ ID NO: 11 - DNA, 34 bp, synthetic construct
  source 1..34: mol_type = other DNA
tgcagcccgggggatcccagccgaagttttaggt

SEQ ID NO: 12 - DNA, 34 bp, synthetic construct
  source 1..34: mol_type = other DNA
tatcggtttcgaatttgggtcagatgtagtcata

SEQ ID NO: 13 - DNA, 36 bp, synthetic construct
  source 1..36: mol_type = other DNA
cggtacccggggatccctcgtgcggaattcgtggag

SEQ ID NO: 14 - DNA, 20 bp, synthetic construct
  source 1..20: mol_type = other DNA
atccagcagcaattcagaca

SEQ ID NO: 15 - DNA, 37 bp, synthetic construct
  source 1..37: mol_type = other DNA
ctgaattgctgctggattaaggcatcgatatcaccca

SEQ ID NO: 16 - DNA, 36 bp, synthetic construct
  source 1..36: mol_type = other DNA
atgcctgcaggtcgacccttcattttaagttccttg

SEQ ID NO: 17 - DNA, 35 bp, synthetic construct
  source 1..35: mol_type = other DNA
cggtacccggggatcctgaccccaggcaagcacgg

SEQ ID NO: 18 - DNA, 27 bp, synthetic construct
  source 1..27: mol_type = other DNA
gaagcgagtacgagtttaagtcttatc

SEQ ID NO: 19 - DNA, 20 bp, synthetic construct
  source 1..20: mol_type = other DNA
aaactcgtactcgcttctcc

SEQ ID NO: 20 - DNA, 35 bp, synthetic construct
  source 1..35: mol_type = other DNA
atgcctgcaggtcgaccggcgccggcaacctcgtc

SEQ ID NO: 21 - DNA, 33 bp, synthetic construct
  source 1..33: mol_type = other DNA
cggtacccggggatccttcatcgatagggtggg

SEQ ID NO: 22 - DNA, 34 bp, synthetic construct
  source 1..34: mol_type = other DNA
gtactcctcagcttactcatcctttgcatcaaca

SEQ ID NO: 23 - DNA, 34 bp, synthetic construct
  source 1..34: mol_type = other DNA
agtaagctgaggagtactgcctgccaaccatcaa

SEQ ID NO: 24 - DNA, 34 bp, synthetic construct
  source 1..34: mol_type = other DNA
atgcctgcaggtcgaccgactggcttgccaccct

SEQ ID NO: 25 - DNA, 40 bp, synthetic construct
  source 1..40: mol_type = other DNA
tgaattcgagctcggtaccccactggtgaactccttgtcc

SEQ ID NO: 26 - DNA, 40 bp, synthetic construct
  source 1..40: mol_type = other DNA
ttgaactaggggcgctttaaaagttttccggtgttgacgg

SEQ ID NO: 27 - DNA, 40 bp, synthetic construct
  source 1..40: mol_type = other DNA
ccgtcaacaccggaaaacttttaaagcgcccctagttcaa

SEQ ID NO: 28 - DNA, 40 bp, synthetic construct
  source 1..40: mol_type = other DNA
gtcgactctagaggatcccccgttgaactgcttgccagcc

SEQ ID NO: 29 - DNA, 40 bp, synthetic construct
  source 1..40: mol_type = other DNA
tgaattcgagctcggtaccctgcggctcgcacggttgctc

SEQ ID NO: 30 - DNA, 40 bp, synthetic construct
  source 1..40: mol_type = other DNA
acggtgcgcaagaagaccacgtcggcagcaaaagcagcct

SEQ ID NO: 31 - DNA, 40 bp, synthetic construct
  source 1..40: mol_type = other DNA
ggctgcttttgctgccgacgtggtcttcttgcgcaccgtg

SEQ ID NO: 32 - DNA, 40 bp, synthetic construct
  source 1..40: mol_type = other DNA
gtcgactctagaggatccccctcttatcaggccaatcggt

SEQ ID NO: 33 - DNA, 42 bp, synthetic construct
  source 1..42: mol_type = other DNA
gtgaattcgagctcggtacccgccccgaaaagccgttaaaag

SEQ ID NO: 34 - DNA, 42 bp, synthetic construct
  source 1..42: mol_type = other DNA
tgccaaaattcacgattattgctcgagtctagagacgggtta

SEQ ID NO: 35 - DNA, 42 bp, synthetic construct
  source 1..42: mol_type = other DNA
ttattggaggagatcaaaacaatgacaatcaaggttgcaatc

SEQ ID NO: 36 - DNA, 42 bp, synthetic construct
  source 1..42: mol_type = other DNA
caggtcggcgtcgcaccttaaggggatcctctagagtcgacc

SEQ ID NO: 37 - DNA, 21 bp, synthetic construct
  source 1..21: mol_type = other DNA
caataatcgtgaattttggca

SEQ ID NO: 38 - DNA, 34 bp, synthetic construct
  source 1..34: mol_type = other DNA
tgttttgatctcctccaataatctatgcttttgc

SEQ ID NO: 39 - DNA, 86 bp, synthetic construct
  source 1..86: mol_type = other DNA
caataatcgtgaattttggcagcaacagaattatgtggtataatggaaacgtgcaaaagcatagattattggaggagatcaaaaca

SEQ ID NO: 40 - DNA, 2196 bp, synthetic construct
  source 1..2196: mol_type = other DNA
atgagttcttctcttaaaattgcttcgactcaagaagcgcgtcaatatttcgatactgaccgcgttgttgtcgatgctgtaggctctgattttactgatgtcggtgctgttatcgcaatggattacgaaacagatgtcatcgacgctgctgatgcaactaagtttggtattcctgtttttgccgtaactaaggatgcccaagctatcagtgctgatgagctgaagaagattttccacatcattgatttggaaaacaaatttgatgctactgttaacgctcgtgaaatcgaaactgctgttaacaactacgaagacagcattttaccaccattcttcaagtcattgaaagaatacgttagccgtggtttaatccaattcgactgcccaggtcaccaaggtggtcaatactacagaaagcacccagctggtcgtgaattctacgacttcttcggcgaaactgtcttccgtgcagacttatgtaacgctgacgttgccttgggtgacttgctgatccacgaaggtcctgctgttgctgctgaaaagcatgctgcacgtgtttacaacgctgacaagacttacttcgttttaggtggttcttccaacgctaacaacactgtaacatctgctttagtttctaacggcgacttggtattgttcgaccggaacaaccacaagtccgtttacaactcagctttagctatggctggtggccgtcctgtttacctccaaacaaaccgtaacccatacggcttcatcggtggtatctacgacagcgacttcgatgaaaagaagatccgtgaactggcagctaaggttgacccagaacgtgctaagtggaagcgtccattccgtctggctgttatccaattaggtacttacgatggtactatctacaacgcacacgaagttgtaaagcgtatcggtcacctttgtgattacatcgaattcgactctgcttgggtaggttacgaacaattcattcctatgatgcgtaactcttcaccattattgattgatgaccttggtccagaagatcctggtatcattgttgttcaatcagttcacaagcaacaagccggcttctcacaaacttcacaaatccacaagaaggatagccacatcaagggtcaattacgttactgtgaccacaagcactttaacaactccttcaacttgttcatgtctacttcaccattctacccaatgtatgcagcattagacgttaacgctgctatgcaagaaggcgaagcaggtcgcaagttatggcatgaccttctgattactaccattgaagctcgtaagaagttgatcaaggctggctcaatgttccgtccattcgttccacctgttgttaacggcaagaagtgggaagatggcgacactgaagatatggctaacaacattgactactggcgctttgaaaagggtgctaagtggcatgcttacgaaggctacggcgacaaccaatactacgttgatccaaacaagttcatgttaactacacctggtatcaacccagaaactggtgactacgaagacttcggtgttccagctactatcgttgctaactacttacgtgaccacggtatcatccctgaaaagtctgacttgaactctatcttgttcttgatgactccagctgaaactccagctaagatgaacaacctgatcactcaacttcttcaattacaacgcttgatcgaagaagatgctccattgaagcaagttcttccttcaatctacgctgctaacgaagaacgttacaatggctacactatccgtgaactttgccaagaattgcacgacttctacaagaacaacaacacgttcacataccagaagcgtctcttcttacgtgaattcttcccagaacaaggtatgcttccatacgaagctcgtcaagaattcatccgcaaccacaacaagcttgttccattgaacaagatcgaaggcgaaatcgccctcgaaggtgctcttccataccctccaggagtattctgtgtagcaccaggtgaaaagtggtcagaaactgctgttaagtacttcactatcttacaagatggtatcaacaacttccctggattcgctccagaaatccaaggtgtatacttcaagcaagaaggcgacaaggttgttgcttacggtgaagtttacgatgcagaagttgctaagaacgatgatcgttacaacaactaa

SEQ ID NO: 41 - DNA, 2196 bp, synthetic construct
  source 1..2196: mol_type = other DNA
atgtcctcttcacttaaaattgcctcgacccaagaagctcgtcagtatttcgataccgaccgtgtggttgtagacgcagttggatccgacttcactgatgtgggagcagtaattgccatggactacgagaccgacgtaattgacgctgcagacgcaaccaaatttggaatcccggtattcgctgtaactaaggacgctcaggcaatttcggccgacgagcttaagaagatctttcacattattgacctcgaaaataagttcgatgctacggtaaacgcccgcgaaattgagactgcagtcaataactacgaagattctatccttccccctttttttaagtcccttaaggagtacgtctcacgcggacttattcagttcgactgcccaggccatcaaggtggacagtactatcggaaacatcccgctggtcgcgaattttacgactttttcggtgaaacggtcttccgtgccgacctctgcaacgcggatgttgcccttggtgaccttctcattcatgagggacccgcggtcgccgctgaaaagcacgcggcacgtgtctacaatgccgacaaaacctattttgtcttgggaggaagctcgaacgctaataacactgtaacttccgccctggtgtccaacggcgacttggtgctgttcgatcgtaataaccataaaagcgtgtacaactcggcacttgcaatggcgggaggtcggcccgtatatttgcagactaatcgtaatccttatggttttattggaggcatctatgattcggattttgacgaaaaaaaaatccgtgaattggctgcgaaggtcgatcctgaacgtgctaaatggaagcgtccgttccggctggctgtgattcagctgggaacttacgacggaactatctataacgcacatgaagtggtgaagcgtatcggtcatttgtgcgactatatcgaattcgattcagcctgggtcggctatgaacagtttatccctatgatgcgcaattcctccccgcttcttatcgacgacctgggtccagaagaccccggaatcattgtagtccaatcggttcataagcagcaagcaggtttctcgcagactagccagattcacaaaaaagactcgcatattaaaggacagcttcggtactgtgaccataagcattttaataacagcttcaacttgttcatgtctaccagccctttttaccctatgtacgcagcactcgacgtaaacgcggcaatgcaggaaggagaggcaggtcggaaactctggcacgatctcttgattacgacgatcgaagcccggaaaaaactcatcaaagctggttccatgttccgtccatttgtaccacctgttgtgaatggtaagaaatgggaagatggagatactgaggatatggccaataacattgattactggcgtttcgaaaaaggtgcgaagtggcatgcatatgaaggctacggcgataatcaatattatgtcgacccaaacaagtttatgttgactactcctggaattaatccggagactggtgattacgaagacttcggcgttcctgcaactatcgttgctaattatcttcgtgaccacggcatcattccagaaaaatccgacctgaatagcattctttttctcatgacccccgcggagacgccggcgaaaatgaataacctgattacgcagttgctgcaactccaacggctcattgaggaggatgctccgcttaaacaagtactgccttcaatttatgccgctaacgaagagcggtataatggatacactatccgtgagctgtgccaggagttgcacgatttttacaagaacaacaatacgttcacctaccagaaacgcctcttcttgcgtgaattttttcccgaacagggaatgttgccatatgaggcgcgtcaagaatttattcgcaaccacaacaagttggttcccctgaacaaaattgaaggcgaaattgccctcgagggcgcgctgccttatcctcctggcgtcttctgtgtggctcctggagagaaatggtcagaaacggcagtgaagtattttaccatccttcaggacggcattaataattttccaggattcgcgcccgagatccaaggtgtgtacttcaagcaggagggagacaaagtagtattgtatggtgaagtgtacgatgcagaagttgccaaaaatgacgaccggtataataattaa

SEQ ID NO: 42 - DNA, 37 bp, synthetic construct
  source 1..37: mol_type = other DNA
gaaaggaaacactcatgtcctcttcacttaaaattgc

SEQ ID NO: 43 - DNA, 39 bp, synthetic construct
  source 1..39: mol_type = other DNA
cttaaatcgccttcagggttaattattataccggtcgtc

SEQ ID NO: 44 - DNA, 32 bp, synthetic construct
  source 1..32: mol_type = other DNA
cgctattctggtatccagaaacatcccagcgc

SEQ ID NO: 45 - DNA, 38 bp, synthetic construct
  source 1..38: mol_type = other DNA
ttttaagtgaagaggacatgagtgtttcctttcgttgg

SEQ ID NO: 46 - DNA, 37 bp, synthetic construct
  source 1..37: mol_type = other DNA
agctcggtacccggggatcccaggaatacagctgttc

SEQ ID NO: 47 - DNA, 34 bp, synthetic construct
  source 1..34: mol_type = other DNA
ctgggatgtttctggataccagaatagcgaaatg

SEQ ID NO: 48 - DNA, 39 bp, synthetic construct
  source 1..39: mol_type = other DNA
gacgaccggtataataattaaccctgaaggcgatttaag

SEQ ID NO: 49 - DNA, 34 bp, synthetic construct
  source 1..34: mol_type = other DNA
gcctgcaggtcgactctagaaatggcagagttgg

SEQ ID NO: 50 - DNA, 5930 bp, synthetic construct
  source 1..5930: mol_type = other DNA
cggctggctggtttattgctgataaatctggagccggtgagcgtgggtctcgcggtatcattgcagcactggggccagatggtaagccctcccgtatcgtagttatctacacgacggggagtcaggcaactatggatgaacgaaatagacagatcgctgagataggtgcctcactgattaagcattggtaactgtcagaccaagtttactcatatatactttagattgatttaaaacttcatttttaatttaaaaggatctaggtgaagatcctttttgataatctcatgaccaaaatcccttaacgtgagttttcgttccactgagcgtcagaccccttaataagatgatcttcttgagatcgttttggtctgcgcgtaatctcttgctctgaaaacgaaaaaaccgccttgcagggcggtttttcgaaggttctctgagctaccaactctttgaaccgaggtaactggcttggaggagcgcagtcaccaaaacttgtcctttcagtttagccttaaccggcgcatgacttcaagactaactcctctaaatcaattaccagtggctgctgccagtggtgcttttgcatgtctttccgggttggactcaagacgatagttaccggataaggcgcagcggtcggactgaacggggggttcgtgcatacagtccagcttggagcgaactgcctacccggaactgagtgtcaggcgtggaatgagacaaacgcggccataacagcggaatgacaccggtaaaccgaaaggcaggaacaggagagcgcacgagggagccgccagggggaaacgcctggtatctttatagtcctgtcgggtttcgccaccactgatttgagcgtcagatttcgtgatgcttgtcaggggggcggagcctatggaaaaacggctttgccgcggccctctcacttccctgttaagtatcttcctggcatcttccaggaaatctccgccccgttcgtaagccatttccgctcgccgcagtcgaacgaccgagcgtagcgagtcagtgagcgaggaagcggaatatatcctgtatcacatattctgctgacgcaccggtgcagccttttttctcctgccacatgaagcacttcactgacaccctcatcagtgccaacatagtaagccagtatacactccgctagcgctgaggtctgcctcgtgaagaaggtgttgctgactcataccaggcctgaatcgccccatcatccagccagaaagtgagggagccacggttgatgagagctttgttgtaggtggaccagttggtgattttgaacttttgctttgccacggaacggtctgcgttgtcgggaagatgcgtgatctgatccttcaactcagcaaaagttcgatttattcaacaaagccacgttgtgtctcaaaatctctgatgttacattgcacaagataaaaatatatcatcatgaacaataaaactgtctgcttacataaacagtaatacaaggggtgttatgagccatattcaacgggaaacgtcttgctcgaggccgcgattaaattccaacatggatgctgatttatatgggtataaatgggctcgcgataatgtcgggcaatcaggtgcgacaatctatcgattgtatgggaagcccgatgcgccagagttgtttctgaaacatggcaaaggtagcgttgccaatgatgttacagatgagatggtcagactaaactggctgacggaatttatgcctcttccgaccatcaagcattttatccgtactcctgatgatgcatggttactcaccactgcgatccccgggaaaacagcattccaggtattagaagaatatcctgattcaggtgaaaatattgttgatgcgctggcagtgttcctgcgccggttgcattcgattcctgtttgtaattgtccttttaacagcgatcgcgtatttcgtctcgctcaggcgcaatcacgaatgaataacggtttggttgatgcgagtgattttgatgacgagcgtaatggctggcctgttgaacaagtctggaaagaaatgcataagcttttgccattctcaccggattcagtcgtcactcatggtgatttctcacttgataaccttatttttgacgaggggaaattaataggttgtattgatgttggacgagtcggaatcgcagaccgataccaggatcttgccatcctatggaactgcctcggtgagttttctccttcattacagaaacggctttttcaaaaatatggtattgataatcctgatatgaataaattgcagtttcatttgatgctcgatgagtttttctaatcagaattggttaattggttgtaacactggcagagcattacgctgacttgacgggacggcggctttgttgaataaatcgaacttttgctgagttgaaggatcagatcacgcatcttcccgacaacgcagaccgttccgtggcaaagcaaaagttcaaaatcaccaactggtccacctacaacaaagctctcatcaaccgtggctccctcactttctggctggatgatggggcgattcaggcctggtatgagtcagcaacaccttcttcacgaggcagacctcagcgctcaaagatgcaggggtaaaagctaaccgcatctttaccgacaaggcatccggcagttcaacagatcgggaagggctggatttgctgaggatgaaggtggaggaaggtgatgtcattctggtgaagaagctcgaccgtcttggccgcgacaccgccgacatgatccaactgataaaagagtttgatgctcagggtgtagcggttcggtttattgacgacgggatcagtaccgacggtgatatggggcaaatggtggtcaccgcgcgtaatacgactcactatagggcgaattggagctccaccgcggtggcggccgctctagaactagtggatcccccgggctgcaggaattcgatatcaagcttatcgataccgtcgacctcgagggggggcccggtacccagcttttgttccctttagtgagggttaattgcgcggtcaccatcctgtcggctgtggcacaggctgaacgccggaggatcagtactgcggcgtcgctgatcgccctcgcgacgttgtgcgggtggcttgtccctgagggcgctgcgacagatagctaaaaatctgcgtcaggatcgccgtagagcgcgcgtcgcgtcgattggaggcttcccctttggttgacggtcttcaatcgctctacggcgatcctgacgcttttttgttgcgtaccgtcgatcgttttatttctgtcgatcccgaaaaagtttttgccttttgtaaaaaacttctcggtcgccccgcaaattttcgattccagattttttaaaaaccaagccagaaatacgacacaccgtttgcagataatctgtctttcggaaaaatcaagtgcgatacaaaatttttagcacccctgagctgcgcaaagtcccgcttcgtgaaaattttcgtgccgcgtgattttccgccaaaaactttaacgaacgttcgttataatggtgtcatgaccttcacgacgaagtaccaaaattggcccgaatcatcagctatggatctctctgatgtcgcgctggagtccgacgcgctcgatgctgccgtcgatttaaaaacggtgatcggatttttccgagctctcgatacgacggacgcgccagcatcacgagactgggccagtgccgcgagcgacctagaaactctcgtggcggatcttgaggagctggctgacgagctgcgtgctcggcagcgccaggaggacgcacagtagtggaggatcgaatcagttgcgcctactgcggtggcctgattcctccccggcctgacccgcgaggacggcgcgcaaaatattgctcagatgcgtgtcgtgccgcagccagccgcgagcgcgccaacaaacgccacgccgaggagctggaggcggctaggtcgcaaatggcgctggaagtgcgtcccccgagcgaaattttggccatggtcgtcacagagctggaagcggcagcgagaattatccgcgatcgtggcgcggtgcccgcaggcatgacaaacatcgtaaatgccgcgtttcgtgtggccgtggccgcccaggacgtgtcagcgccgccaccacctgcaccgaatcggcagcagcgtcgcgcgtcgaaaaagcgcacaggcggcaagaagcgataagctgcacgaatacctgaaaaatgttgaacgccccgtgagcggtaactcacagggcgtcggctaacccccagtccaaacctgggagaaagcgctcaaaaatgactctagcggattcacgagacattgacacaccggcctggaaattttccgctgatctgttcgacacccatcccgagctcgcgctgcgatcacgtggctggacgagcgaagaccgccgcgaattcctcgctcacctgggcagagaaaatttccagggcagcaagacccgcgacttcgccagcgcttggatcaaagacccggacacgggagaaacacagccgaagttataccgagttggttcaaaatcgcttgcccggtgccagtatgttgctctgacgcacgcgcagcacgcagccgtgcttgtcctggacattgatgtgccgagccaccaggccggcgggaaaatcgagcacgtaaaccccgaggtctacgcgattttggagcgctgggcacgcctggaaaaagcgccagcttggatcggcgtgaatccactgagcgggaaatgccagctcatctggctcattgatccggtgtatgccgcagcaggcatgagcagcccgaatatgcgcctgctggctgcaacgaccgaggaaatgacccgcgttttcggcgctgaccaggctttttcacataggctgagccggtggccactgcacgtctccgacgatcccaccgcgtaccgctggcatgcccagcacaatcgcgtggatcgcctagctgatcttatggaggttgctcgcatgatctcaggcacagaaaaacctaaaaaacgctatgagcaggagttttctagcggacgggcacgtatcgaagcggcaagaaaagccactgcggaagcaaaagcacttgccacgcttgaagcaagcctgccgagcgccgctgaagcgtctggagagctgatcgacggcgtccgtgtcctctggactgctccagggcgtgccgcccgtgatgagacggcttttcgccacgctttgactgtgggataccagttaaaagcggctggtgagcgcctaaaagacaccaagatcatcgacgcctacgagcgtgcctacaccgtcgctcaggcggtcggagcagacggccgtgagcctgatctgccgccgatgcgtgaccgccagacgatggcgcgacgtgtgcgcggctacgtcgctaaaggccagccagtcgtccctgctcgtcagacagagacgcagagcagccgagggcgaaaagctctggccactatgggaagacgtggcggtaaaaaggccgcagaacgctggaaagacccaaacagtgagtacgcccgagcacagcgagaaaaactagctaagtccagtcaacgacaagctaggaaagctaaaggaaatcgcttgaccattgcaggttggtttatgactgttgagggagagactggctcgtggcgacaatcaatgaagctatgtctgaatttagcgtgtcacgtcagaccgtgaatagagcacttaagtctgcgggcattgaacttccacgaggacgccgtaaagcttcccagtaaatgtgccatctcgtaggcagaaaacggttccccccgtaggggtctctctcttggcctcctttctaggtcgggctgattgctcttgaagctctctaggggggctcacaccataggcagataacggttccccaccggctcacctcgtaagcgcacaaggactgctcccaaagatc

SEQ ID NO: 51 - DNA, 5802 bp, synthetic construct
  source 1..5802: mol_type = other DNA
gttcgcttgctgtccataaaaccgcccagtctagctatcgccatgtaagcccactgcaagctacctgctttctctttgcgcttgcgttttcccttgtccagatagcccagtagctgacattcatccggggtcagcaccgtttctgcggactggctttctacgtgttccgcttcctttagcagcccttgcgccctgagtgcttgcggcagcgtgaagctagcttttatcgccattcgccattcaggctgcgcaactgttgggaagggcgatcggtgcgggcctcttcgctattacgccagctggcgaaagggggatgtgctgcaaggcgattaagttgggtaacgccagggttttcccagtcacgacgttgtaaaacgacggccagtgaattcgagctcggtacccggggatcctctagagtcgacctgcaggcatgcaagcttggcgtaatcatggtcatagctgtttcctgtgtgaaattgttatccgctcacaattccacacaacatacgagccggaagcataaagtgtaaagcctggggtgcctaatgagtgagctaactcacattaattgcgttgcgctcactgcccgctttccagtcgggaaacctgtcgtgccagctgcattaatgaatcggccaacgcgcggggagaggcggtttgcgtattgggcgctcttccgcttcctcgctcactgactcgctgcgctcggtcgttcggctgcggcgagcggtatcagctcactcaaaggcggtaatacggttatccacagaatcaggggataacgcaggaaagaacatgtgagcaaaaggccagcaaaaggccaggaaccgtaaaaaggccgcgttgctggcgtttttccataggctccgcccccctgacgagcatcacaaaaatcgacgctcaagtcagaggtggcgaaacccgacaggactataaagataccaggcgtttccccctggaagctccctcgtgcgctctcctgttccgaccctgccgcttaccggatacctgtccgcctttctcccttcgggaagcgtggcgctttctcaatgctcacgctgtaggtatctcagttcggtgtaggtcgttcgctccaagctgggctgtgtgcacgaaccccccgttcagcccgaccgctgcgccttatccggtaactatcgtcttgagtccaacccggtaagacacgacttatcgccactggcagcagccactggtaacaggattagcagagcgaggtatgtaggcggtgctacagagttcttgaagtggtggcctaactacggctacactagaaggacagtatttggtatctgcgctctgctgaagccagttaccttcggaaaaagagttggtagctcttgatccggcaaacaaaccaccgctggtagcggtggtttttttgtttgcaagcagcagattacgcgcagaaaaaaaggatctcaagaagatcctttgatcttttctacggggtctgacgctcagtggaacgaaaactcacgttaagggattttggtcatgagattatcaaaaaggatcttcacctagatccttttggggtgggcgaagaactccagcatgagatccccgcgctggaggatcatccagccctgatagaaacagaagccactggagcacctcaaaaacaccatcatacactaaatcagtaagttggcagcatcacccgacgcactttgcgccgaataaatacctgtgacggaagatcacttcgcagaataaataaatcctggtgtccctgttgataccgggaagccctgggccaacttttggcgaaaatgagacgttgatcggcacgtaagaggttccaactttcaccataatgaaataagatcactaccgggcgtattttttgagttatcgagattttcaggagctgatagaaacagaagccactggagcacctcaaaaacaccatcatacactaaatcagtaagttggcagcatcacccgacgcactttgcgccgaataaatacctgtgacggaagatcacttcgcagaataaataaatcctggtgtccctgttgataccgggaagccctgggccaacttttggcgaaaatgagacgttgatcggcacgtaagaggttccaactttcaccataatgaaataagatcactaccgggcgtattttttgagttatcgagattttcaggagctctttggcatcgtctctcgcctgtcccctcagttcagtaatttcctgcatttgcctgtttccagtcggtagatattccacaaaacagcagggaagcagcgcttttccgctgcataaccctgcttcggggtcattatagcgattttttcggtatatccatcctttttcgcacgatatacaggattttgccaaagggttcgtgtagactttccttggtgtatccaacggcgtcagccgggcaggataggtgaagtaggcccacccgcgagcgggtgttccttcttcactgtcccttattcgcacctggcggtgctcaacgggaatcctgctctgcgaggctggccggctaccgccggcgtaacagatgagggcaagcggatggctgatgaaaccaagccaaccaggaagggcagcccacctatcaaggtgtactgccttccagacgaacgaagagcgattgaggaaaaggcggcggcggccggcatgagcctgtcggcctacctgctggccgtcggccagggctacaaaatcacgggcgtcgtggactatgagcacgtccgcgagggcgtcccggaaaacgattccgaagcccaacctttcatagaaggcggcggtggaatcgaaatctcgtgatggcaggttgggcgtcgcttggtcggtcatttcgaaaaaggttaggaatacggttagccatttgcctgcttttatatagttcatatgggattcacctttatgttgataagaaataaaagaaaatgccaataggatatcggcattttcttttgcgtttttatttgttaactgttaattgtccttgttcaaggatgctgtctttgacaacagatgttttcttgcctttgatgttcagcaggaagctcggcgcaaacgttgattgtttgtctgcgtagaatcctctgtttgtcatatagcttgtaatcacgacattgtttcctttcgcttgaggtacagcgaagtgtgagtaagtaaaggttacatcgttaggcggatcaagatccatttttaacacaaggccagttttgttcagcggcttgtatgggccagttaaagaattagaaacataaccaagcatgtaaatatcgttagacgtaatgccgtcaatcgtcatttttgatccgcgggagtcagtgaacaggtaccatttgccgttcattttaaagacgttcgcgcgttcaatttcatctgttactgtgttagatgcaatcagcggtttcatcacttttttcagtgtgtaatcatcgtttagctcaatcataccgagagcgccgtttgctaactcagccgtgcgttttttatcgctttgcagaagtttttgactttcttgacggaagaatgatgtgcttttgccatagtatgctttgttaaataaagattcttcgccttggtagccatcttcagttccagtgtttgcttcaaatactaagtatttgtggcctttatcttctacgtagtgaggatctctcagcgtatggttgtcgcctgagctgtagttgccttcatcgatgaactgctgtacattttgatacgtttttccgtcaccgtcaaagattgatttataatcctctacaccgttgatgttcaaagagctgtctgatgctgatacgttaacttgtgcagttgtcagtgtttgtttgccgtaatgtttaccggagaaatcagtgtagaataaacggatttttccgtcagatgtaaatgtggctgaacctgaccattcttgtgtttggtcttttaggatagaatcatttgcatcgaatttgtcgctgtctttaaagacgcggccagcgtttttccagctgtcaatagaagtttcgccgactttttgatagaacatgtaaatcgatgtgtcatccgcatttttaggatctccggctaatgcaaagacgatgtggtagccgtgatagtttgcgacagtgccgtcagcgttttgtaatggccagctgtcccaaacgtccaggccttttgcagaagagatatttttaattgtggacgaatcaaattcagaaacttgatatttttcatttttttgctgttcagggatttgcagcatatcatggcgtgtaatatgggaaatgccgtatgtttccttatatggcttttggttcgtttctttcgcaaacgcttgagttgcgcctcctgccagcagtgcggtagtaaaggttaatactgttgcttgttttgcaaactttttgatgttcatcgttcatgtctccttttttatgtactgtgttagcggtctgcttcttccagccctcctgtttgaagatggcaagttagttacgcacaataaaaaaagacctaaaatatgtaaggggtgacgccaaagtatacactttgccctttacacattttaggtcttgcctgctttatcagtaacaaacccgcgcgatttacttttcgacctcattctattagactctcgtttggattgcaactggtctattttcctcttttgtttgatagaaaatcataaaaggatttgcagactacgggcctaaagaactaaaaaatctatctgtttcttttcattctctgtattttttatagtttctgttgcatgggcataaagttgcctttttaatcacaattcagaaaatatcataatatctcatttcactaaataatagtgaacggcaggtatatgtgatgggttaaaaaggatcaccccagagtcccgctcagaagaactcgtcaagaaggcgatagaaggcgatgcgctgcgaatcgggagcggcgataccgtaaagcacgaggaagcggtcagcccattcgccgccaagctcttcagcaatatcacgggtagccaacgctatgtcctgatagcggtccgccacacccagccggccacagtcgatgaatccagaaaagcggccattttccaccatgatattcggcaagcaggcatcgccatgggtcacgacgagatcctcgccgtcgggcatccgcgccttgagcctggcgaacagttcggctggcgcgagcccctgatgctcttcgtccagatcatcctgatcgacaagaccggcttccatccgagtacgtgctcgctcgatgcgatgtttcgcttggtggtcgaatgggcaggtagccggatcaagcgtatgcagccgccgcattgcatcagccatgatggatactttctcggcaggagcaaggtgagatgacaggagatcctgccccggcacttcgcccaatagcagccagtcccttcccgcttcagtgacaacgtcgagacagctgcgcaaggaacgcccgtcgtggccagccacgatagccgcgctgcctcgtcttggagttcattcagggcaccggacaggtcggtcttgacaaaaagaaccgggcgcccctgcgctgacagccggaacacggcggcatcagagcagccgattgtctgttgtgcccagtcatagccgaatagcctctccacccaagcggccggagaacctgcgtgcaatccatcttgttcaatcatgcgaaacgatcctcatcctgtctcttgatcagatcttgatcccctgcgccatcagatccttggcggcaagaaagccatccagtttactttgcagggcttcccaaccttaccagagggcgccccagctggcaattccg

SEQ ID NO: 52 - DNA, 612 bp, synthetic construct
  source 1..612: mol_type = other DNA
atgagtcccaccgttttgcctgctacacaagctgacttccctaagatcgtcgatgttctggttgaagcattcgccaacgatccagcatttttacgatggatcccgcagccggaccccggttcagcaaagcttcgagcacttttcgaactgcagattgagaagcagtatgcagtggcgggaaatattgatgtcgcgcgtgattctgagggagaaatcgtcggcgtcgcgttatgggatcggccagatggtaatcacagtgccaaagatcaagcagcgatactcccccggctcgtctccattttcgggatcaaggctgcgcaggtggcgtggacggatttgagttcggctcgtttccaccccaaattcccccattggtacctctacaccgtggcaacatctagttctgcccgtggaacgggtgttggcagtgcgcttcttaatcacggaatcgctcgcgcgggtgatgaagctatctatttggaggcgacgtcgactcgtgcggctcaactatataaccgtctgggatttgtgcccttgggttatatcccctcagatgatgatggcactcctgaactggcgatgtggaaaccgccagcgatgccaactgtttaa